European Patent Application EP 4 603 481 A1, published August 20, 2025. Title: 一种阳离子脂质材料的制备及应用. Applicant: 南京吉迈生物技术有限公司. Application WO. The sequence listing filed with the application follows.

SEQUENCE LISTING (2 sequences)

SEQ ID NO: 1 - RNA, 2008 nt, synthetic construct
  source 1..2008: mol_type = other RNA
agggaaataagagagaaaagaagagtaagaacagggcagagccatctattgcttacatttgcttctgacacaactgtgttcactagcaacctcaaacagacaccatggaggacgccaagaacatcaagaagggccccgcccccttctaccccctggaggacggcaccgccggcgagcagctgcacaaggccatgaagcggtacgccctggtgcccggcaccatcgccttcaccgacgcccacatcgaggtggacatcacctacgccgagtacttcgagatgagcgtgcggctggccgaggccatgaagcggtacggcctgaacaccaaccaccggatcgtggtgtgcagcgagaacagcctgcagttcttcatgcccgtgctgggcgccctgttcatcggcgtggccgtggcccccgccaacgacatctacaacgagcgggagctgctgaacagcatgggcatcagccagcccaccgtggtgttcgtgagcaagaagggcctgcagaagatcctgaacgtgcagaagaagctgcccatcatccagaagatcatcatcatggacagcaagaccgactaccagggcttccagagcatgtacaccttcgtgaccagccacctgccccccggcttcaacgagtacgacttcgtgcccgagagcttcgaccgggacaagaccatcgccctgatcatgaacagcagcggcagcaccggcctgcccaagggcgtggccctgccccaccggaccgcctgcgtgcggttcagccacgcccgggaccccatcttcggcaaccagatcatccccgacaccgccatcctgagcgtggtgcccttccaccacggcttcggcatgttcaccaccctgggctacctgatctgcggcttccgggtggtgctgatgtaccggttcgaggaggagctgttcctgcggagcctgcaggactacaagatccagagcgccctgctggtgcccaccctgttcagcttcttcgccaagagcaccctgatcgacaagtacgacctgagcaacctgcacgagatcgccagcggcggcgcccccctgagcaaggaggtgggcgaggccgtggccaagcggttccacctgcccggcatccggcagggctacggcctgaccgagaccaccagcgccatcctgatcacccccgagggcgacgacaagcccggcgccgtgggcaaggtggtgcccttcttcgaggccaaggtggtggacctggacaccggcaagaccctgggcgtgaaccagcggggcgagctgtgcgtgcggggccccatgatcatgagcggctacgtgaacaaccccgaggccaccaacgccctgatcgacaaggacggctggctgcacagcggcgacatcgcctactgggacgaggacgagcacttcttcatcgtggaccggctgaagagcctgatcaagtacaagggctaccaggtggcccccgccgagctggagagcatcctgctgcagcaccccaacatcttcgacgccggcgtggccggcctgcccgacgacgacgccggcgagctgcccgccgccgtggtggtgctggagcacggcaagaccatgaccgagaaggagatcgtggactacgtggccagccaggtgaccaccgccaagaagctgcggggcggcgtggtgttcgtggacgaggtgcccaagggcctgaccggcaagctggacgcccggaagatccgggagatcctgatcaaggccaagaagggcggcaagatcgccgtgtgatgatagtaagctcgctttcttgctgtccaatttctattaaaggttcctttgttccctaagtccaactactaaactgggggatattatgaagggccttgagcatctggattctgcctaataaaaaacatttattttcattgcaaaaaaaaaaaaaaaaaaaaaaaaaaaaaagcatatgactaaaaaaaaaaaaaaaaaaaaaaaaaaaaaaaaaaaaaaaaaaaaaaaaaaaaaaaaaaaaaaaaaaaaaa

SEQ ID NO: 2 - RNA, 1107 nt, synthetic construct
  source 1..1107: mol_type = other RNA
aggtgtatttactagtaacgtaacagtgttacgtagtgacgtttaactgagactatggactggacctggatcctgttcctggtggccgccgccaccagagtgcacagcttccaggacccccaggagagcggcagaaagctgccccagctgtgcaccgagctgcagaccaccatccacgacatcatcctggagtgcgtgtactgcaagcagcagctgctgagaagagaggtgtacgacagagacctgtgcatcgtgtacagagacggcaacccctacgccgtgtgcgacaagtgcctgaagttctacagcaagatcagcgagtacagacactactgctacagcctgtacggcaccaccctggagcagcagtacaacaagcccctgtgcgacctgctgatcagatgcatcaactgccagaagcccctgcagagacacctggacaagaagcagagattccacaacatcagaggcagatggaccggcagatgcatgagctgctgcagaagcagcagaaccagaagagagacccagctgagaggcagaaagagaagaagccacggcgacacccccaccctgcacgagtacatgctggacctgcagcccgagaccaccgacctgtacggctacggccagctgaacgacagcagcgaggaggaggacgagatcgacggccccgccggccaggccgagcccgacagagcccactacaacatcgtgaccttctgctgcaagtgcgacagcaccctgagactgtgcgtgcagagcacccacgtggacatcagaaccctggaggacctgctgatgggcaccctgggcatcgtgtgccccatctgcagccagaagccctgataataggctcgctttcttgctgtccaatttctattaaaggttcctttgttccctaagtccaactactaaactgggggatattatgaagggccttgagcatctggattctgcctaataaaaaacatttattttcattgcaaaaaaaaaaaaaaaaaaaaaaaaaaaaaaaaaaaaaaaaaaaaaaaaaaaaaaaaaaaaaaaaaaaaaaaaaaaaaaaaaaaaaaaaaaaaaaaaaaaaaaaaaaaaaaaaaaaaaaaa